European Patent Specification EP 3 773 713 B1, published July 9, 2025. Title: METHODS OF TREATMENT USING A LEPTIN RECEPTOR AGONIST ANTIBODY. Applicant: Regeneron Pharmaceuticals, Inc. Gromada, Jesper Stevis, Panayiotis Altarejos, Judith Murphy, Andrew J. Application TBD. The sequence listing filed with the application follows.

SEQUENCE LISTING (120 sequences)

SEQ ID NO: 1 - DNA, 357 bp, Artificial Sequence
  synthetic
caggtgcagctggtggagtctgggggaggcgtggtccagcctgggaagtccctgagactctcctgtgtagcgtctggattcaccttcagttccgatgccatgtactgggtccgccaggctccaggcaaggggctggaatgggtggcagttatttattatgatggaaattatcaatactatgaagactccgttaagggtcgattcaccatctccagagacaattcccagaacacgctggatctgcaaatgaacagcctgagagtcgacgacacggctgtatatttctgtgcgcgtctcaactgggattactggtatctcgatctctggggccgtggcaccctggtcactgtctcctca

SEQ ID NO: 2 - protein, 119 aa, Artificial Sequence
  synthetic
QVQLVESGGGVVQPGKSLRLSCVASGFTFSSDAMYWVRQAPGKGLEWVAVIYYDGNYQYYEDSVKGRFTISRDNSQNTLDLQMNSLRVDDTAVYFCARLNWDYWYLDLWGRGTLVTVSS

SEQ ID NO: 3 - DNA, 24 bp, Artificial Sequence
  synthetic
ggattcaccttcagttccgatgcc

SEQ ID NO: 4 - protein, 8 aa, Artificial Sequence
  synthetic
GFTFSSDA

SEQ ID NO: 5 - DNA, 24 bp, Artificial Sequence
  synthetic
atttattatgatggaaattatcaa

SEQ ID NO: 6 - protein, 8 aa, Artificial Sequence
  synthetic
IYYDGNYQ

SEQ ID NO: 7 - DNA, 36 bp, Artificial Sequence
  synthetic
gcgcgtctcaactgggattactggtatctcgatctc

SEQ ID NO: 8 - protein, 12 aa, Artificial Sequence
  synthetic
ARLNWDYWYLDL

SEQ ID NO: 9 - DNA, 324 bp, Artificial Sequence
  synthetic
gacatccagatgacccagtctccatcctccctgtctgcatctgtaggagacagagtcaccatcacttgccgggcaagtcagagcattagcagctatttaaattggtatcagcagaaaccagggaaagcccctaagctcctgatctatgctgcatccagtttgcaaagtggggtcccgtcaaggttcagtggcagtggatctgggacagatttcactctcaccatcagcagtctgcaacctgaagattttgcaacttactactgtcaacagagttacagtacccctccgatcaccttcggccaagggacacgactggagattaaa

SEQ ID NO: 10 - protein, 108 aa, Artificial Sequence
  synthetic
DIQMTQSPSSLSASVGDRVTITCRASQSISSYLNWYQQKPGKAPKLLIYAASSLQSGVPSRFSGSGSGTDFTLTISSLQPEDFATYYCQQSYSTPPITFGQGTRLEIK

SEQ ID NO: 11 - DNA, 18 bp, Artificial Sequence
  synthetic
cagagcattagcagctat

SEQ ID NO: 12 - protein, 6 aa, Artificial Sequence
  synthetic
QSISSY

SEQ ID NO: 13 - DNA, 9 bp, Artificial Sequence
  synthetic
gctgcatcc

SEQ ID NO: 14 - protein, 3 aa, Artificial Sequence
  synthetic
AAS

SEQ ID NO: 15 - DNA, 30 bp, Artificial Sequence
  synthetic
caacagagttacagtacccctccgatcacc

SEQ ID NO: 16 - protein, 10 aa, Artificial Sequence
  synthetic
QQSYSTPPIT

SEQ ID NO: 17 - DNA, 357 bp, Artificial Sequence
  synthetic
caggtgcagctggtggagtccgggggaggcgtggtccagcctgggaggtccctgagactctcctgtacagcgtctggattcaccttcagtagttatgccatgtactgggtccgccaggctccaggcaaggggctggagtgggtgtcagttatatactatgatggaagttataaatactatgcagactccgtgaagggccgattcaccatctccagagacaattccaagaacacgctgtatctgcaaatggacagcctgagagccgaggacacggctgtctattactgtgcgagttataactggaactactggtacttcgatttctggggccgtggcaccctggtcactgtctcctca

SEQ ID NO: 18 - protein, 119 aa, Artificial Sequence
  synthetic
QVQLVESGGGVVQPGRSLRLSCTASGFTFSSYAMYWVRQAPGKGLEWVSVIYYDGSYKYYADSVKGRFTISRDNSKNTLYLQMDSLRAEDTAVYYCASYNWNYWYFDFWGRGTLVTVSS

SEQ ID NO: 19 - DNA, 24 bp, Artificial Sequence
  synthetic
ggattcaccttcagtagttatgcc

SEQ ID NO: 20 - protein, 8 aa, Artificial Sequence
  synthetic
GFTFSSYA

SEQ ID NO: 21 - DNA, 24 bp, Artificial Sequence
  synthetic
atatactatgatggaagttataaa

SEQ ID NO: 22 - protein, 8 aa, Artificial Sequence
  synthetic
IYYDGSYK

SEQ ID NO: 23 - DNA, 36 bp, Artificial Sequence
  synthetic
gcgagttataactggaactactggtacttcgatttc

SEQ ID NO: 24 - protein, 12 aa, Artificial Sequence
  synthetic
ASYNWNYWYFDF

SEQ ID NO: 25 - DNA, 357 bp, Artificial Sequence
  synthetic
caggtgcagctggtggagtctgggggaagcgtggtccagcctgggaggtccctgagactctcctgtgcagcgtctggattcaccttcagtacatatgccatgtactgggtccgccagactccaggcaaggggctggagtgggtggctgttttatactctgatggaagtaataaatactatatagactccgtgaagggccgattcaccatctccagagacacttccacgaacactctgtatctgcaaatgagcagcctgcgagccgacgactcggctctatattactgtgcgcgtctcaactgggattactggtacttcgatctctggggccgtggcaccctggtcactgtctcctca

SEQ ID NO: 26 - protein, 119 aa, Artificial Sequence
  synthetic
QVQLVESGGSVVQPGRSLRLSCAASGFTFSTYAMYWVRQTPGKGLEWVAVLYSDGSNKYYIDSVKGRFTISRDTSTNTLYLQMSSLRADDSALYYCARLNWDYWYFDLWGRGTLVTVSS

SEQ ID NO: 27 - DNA, 24 bp, Artificial Sequence
  synthetic
ggattcaccttcagtacatatgcc

SEQ ID NO: 28 - protein, 8 aa, Artificial Sequence
  synthetic
GFTFSTYA

SEQ ID NO: 29 - DNA, 24 bp, Artificial Sequence
  synthetic
ttatactctgatggaagtaataaa

SEQ ID NO: 30 - protein, 8 aa, Artificial Sequence
  synthetic
LYSDGSNK

SEQ ID NO: 31 - DNA, 36 bp, Artificial Sequence
  synthetic
gcgcgtctcaactgggattactggtacttcgatctc

SEQ ID NO: 32 - protein, 12 aa, Artificial Sequence
  synthetic
ARLNWDYWYFDL

SEQ ID NO: 33 - DNA, 357 bp, Artificial Sequence
  synthetic
caggtgcagctggtggagtctgggggaggcgtggtccagcctgggaggtccctgagactctcctgtgaagcgtctggattcagcagcagtgacaatgccatgtactgggtccgccaggctccaggcaaggggctggagtgggtgtcagttatatatcatgatggaagttataaatactatgaagactccgtgaagggccgattcaccatcgccagagacaattccaagaacacgctttatttgcaaatgaacagcctgagagccgaggacacggctgtatattactgtgcgaggtataactggaaccactggtacttcgatgtctggggccgtggcaccctggtcactgtctcctca

SEQ ID NO: 34 - protein, 119 aa, Artificial Sequence
  synthetic
QVQLVESGGGVVQPGRSLRLSCEASGFSSSDNAMYWVRQAPGKGLEWVSVIYHDGSYKYYEDSVKGRFTIARDNSKNTLYLQMNSLRAEDTAVYYCARYNWNHWYFDVWGRGTLVTVSS

SEQ ID NO: 35 - DNA, 24 bp, Artificial Sequence
  synthetic
ggattcagcagcagtgacaatgcc

SEQ ID NO: 36 - protein, 8 aa, Artificial Sequence
  synthetic
GFSSSDNA

SEQ ID NO: 37 - DNA, 24 bp, Artificial Sequence
  synthetic
atatatcatgatggaagttataaa

SEQ ID NO: 38 - protein, 8 aa, Artificial Sequence
  synthetic
IYHDGSYK

SEQ ID NO: 39 - DNA, 36 bp, Artificial Sequence
  synthetic
gcgaggtataactggaaccactggtacttcgatgtc

SEQ ID NO: 40 - protein, 12 aa, Artificial Sequence
  synthetic
ARYNWNHWYFDV

SEQ ID NO: 41 - DNA, 366 bp, Artificial Sequence
  synthetic
caggtgcagctggtggagtctgggggaggcgtggtccagcctgggaggtccctgagactctcctgtgcagcctctggattcaccttcagtacctatggcatgcactgggtccgccaggctccaggcaaggggctggagtgggtgtcagttatatcatatgacgaaagtaataagtactatgcagactccgtgaagggccgattcaccatttctagagacaattccaagaacgcgctgtatttacaaatgaacagcctgagaaatgaggacacggctgtgtattactgtgcgagagatcggccttttggattggttaccggatggttcgacccctggggccagggaaccctggtcaccgtctcctca

SEQ ID NO: 42 - protein, 122 aa, Artificial Sequence
  synthetic
QVQLVESGGGVVQPGRSLRLSCAASGFTFSTYGMHWVRQAPGKGLEWVSVISYDESNKYYADSVKGRFTISRDNSKNALYLQMNSLRNEDTAVYYCARDRPFGLVTGWFDPWGQGTLVTVSS

SEQ ID NO: 43 - DNA, 24 bp, Artificial Sequence
  synthetic
ggattcaccttcagtacctatggc

SEQ ID NO: 44 - protein, 8 aa, Artificial Sequence
  synthetic
GFTFSTYG

SEQ ID NO: 45 - DNA, 24 bp, Artificial Sequence
  synthetic
atatcatatgacgaaagtaataag

SEQ ID NO: 46 - protein, 8 aa, Artificial Sequence
  synthetic
ISYDESNK

SEQ ID NO: 47 - DNA, 45 bp, Artificial Sequence
  synthetic
gcgagagatcggccttttggattggttaccggatggttcgacccc

SEQ ID NO: 48 - protein, 15 aa, Artificial Sequence
  synthetic
ARDRPFGLVTGWFDP

SEQ ID NO: 49 - DNA, 360 bp, Artificial Sequence
  synthetic
caggtgcagctggtggagtctgggggaggcgtggtccagcctgggaggtccctgagactctcctgtgcagcgtctggattcagtttcaatacctatggcatgcactgggtccgccaggctccaggcaaggggctggagtgggtgacaattatatggtatgatggaagtattaaatactatgcagactccgtgaagggccgattcaccatctccagagacaattccaagaacacgctgtatctgcaaatgaacagcctgagagccgaggacacggctgtgtattattgtgcgagaggtggatatagtggctacctctactttgactactggggccagggaaccctggtcaccgtctcctca

SEQ ID NO: 50 - protein, 120 aa, Artificial Sequence
  synthetic
QVQLVESGGGVVQPGRSLRLSCAASGFSFNTYGMHWVRQAPGKGLEWVTIIWYDGSIKYYADSVKGRFTISRDNSKNTLYLQMNSLRAEDTAVYYCARGGYSGYLYFDYWGQGTLVTVSS

SEQ ID NO: 51 - DNA, 24 bp, Artificial Sequence
  synthetic
ggattcagtttcaatacctatggc

SEQ ID NO: 52 - protein, 8 aa, Artificial Sequence
  synthetic
GFSFNTYG

SEQ ID NO: 53 - DNA, 24 bp, Artificial Sequence
  synthetic
atatggtatgatggaagtattaaa

SEQ ID NO: 54 - protein, 8 aa, Artificial Sequence
  synthetic
IWYDGSIK

SEQ ID NO: 55 - DNA, 39 bp, Artificial Sequence
  synthetic
gcgagaggtggatatagtggctacctctactttgactac

SEQ ID NO: 56 - protein, 13 aa, Artificial Sequence
  synthetic
ARGGYSGYLYFDY

SEQ ID NO: 57 - DNA, 372 bp, Artificial Sequence
  synthetic
caggtgcagctgcaggagtcgggcccaggactggtgaagccttcacagaccctgtccctcacctgcactgtctctggtggctccatcagcagcggtggtgactactggagctggatccgccagctcccagggaagggcctggagtggattgggtacatctattacagtgggagcgcctactataatccgtccctcaagagtcgaggtaccatatcaatagacacgtctaagaaccagttctccctgaagctgacctctgtgactgccgcggacacggccgtatatttctgtgtgaaattacgatttttggagtggttcttggggggctggttcggcccctggggccagggaaccctggtcaccgtctcctca

SEQ ID NO: 58 - protein, 124 aa, Artificial Sequence
  synthetic
QVQLQESGPGLVKPSQTLSLTCTVSGGSISSGGDYWSWIRQLPGKGLEWIGYIYYSGSAYYNPSLKSRGTISIDTSKNQFSLKLTSVTAADTAVYFCVKLRFLEWFLGGWFGPWGQGTLVTVSS

SEQ ID NO: 59 - DNA, 30 bp, Artificial Sequence
  synthetic
ggtggctccatcagcagcggtggtgactac

SEQ ID NO: 60 - protein, 10 aa, Artificial Sequence
  synthetic
GGSISSGGDY

SEQ ID NO: 61 - DNA, 21 bp, Artificial Sequence
  synthetic
atctattacagtgggagcgcc

SEQ ID NO: 62 - protein, 7 aa, Artificial Sequence
  synthetic
IYYSGSA

SEQ ID NO: 63 - DNA, 48 bp, Artificial Sequence
  synthetic
gtgaaattacgatttttggagtggttcttggggggctggttcggcccc

SEQ ID NO: 64 - protein, 16 aa, Artificial Sequence
  synthetic
VKLRFLEWFLGGWFGP

SEQ ID NO: 65 - DNA, 351 bp, Artificial Sequence
  synthetic
gaggtgcagctggtggagtctgggggaggcttggtacagccgggggggtccctgagactctcctgtgcagcctctggattcacctttagcaactatggcatgacctgggtccgccaggctccagggaagggcctggaatgggtctcagctattactggtggtggtggtagcacatactactcaaactccgtgaagggccggttcaccatctccagagacaattccaagaacacggtgtatctgcgaatgaacagtgtgagagccgaggacacggccgtatattactgtgcgaaatataagtggaacttcgtggacgactggggccagggaaccacggtcaccgtctcctca

SEQ ID NO: 66 - protein, 117 aa, Artificial Sequence
  synthetic
EVQLVESGGGLVQPGGSLRLSCAASGFTFSNYGMTWVRQAPGKGLEWVSAITGGGGSTYYSNSVKGRFTISRDNSKNTVYLRMNSVRAEDTAVYYCAKYKWNFVDDWGQGTTVTVSS

SEQ ID NO: 67 - DNA, 24 bp, Artificial Sequence
  synthetic
ggattcacctttagcaactatggc

SEQ ID NO: 68 - protein, 8 aa, Artificial Sequence
  synthetic
GFTFSNYG

SEQ ID NO: 69 - DNA, 24 bp, Artificial Sequence
  synthetic
attactggtggtggtggtagcaca

SEQ ID NO: 70 - protein, 8 aa, Artificial Sequence
  synthetic
ITGGGGST

SEQ ID NO: 71 - DNA, 30 bp, Artificial Sequence
  synthetic
gcgaaatataagtggaacttcgtggacgac

SEQ ID NO: 72 - protein, 10 aa, Artificial Sequence
  synthetic
AKYKWNFVDD

SEQ ID NO: 73 - DNA, 360 bp, Artificial Sequence
  synthetic
gaggtgcagctggtggagtctgggggaggcttggtacagcctggggggtccctgagactctcctgtgttgcctctggattcaccttcaataaatacgacatgcactgggtccgccaaactactggaaaaggtctagagtgggtctcaggtattgatactgatggtgacacatactatccaggctccgtgaagggccgattcaccatctccagagaaaatgccgagaactccctgtatcttcaaatgaacggcctgagagtcggggacacggctgtgtattactgtgcaagatggccttggagtggtttctatggtgcttttgatatctggggccaagggacaatggtcaccgtctcttca

SEQ ID NO: 74 - protein, 120 aa, Artificial Sequence
  synthetic
EVQLVESGGGLVQPGGSLRLSCVASGFTFNKYDMHWVRQTTGKGLEWVSGIDTDGDTYYPGSVKGRFTISRENAENSLYLQMNGLRVGDTAVYYCARWPWSGFYGAFDIWGQGTMVTVSS

SEQ ID NO: 75 - DNA, 24 bp, Artificial Sequence
  synthetic
ggattcaccttcaataaatacgac

SEQ ID NO: 76 - protein, 8 aa, Artificial Sequence
  synthetic
GFTFNKYD

SEQ ID NO: 77 - DNA, 21 bp, Artificial Sequence
  synthetic
attgatactgatggtgacaca

SEQ ID NO: 78 - protein, 7 aa, Artificial Sequence
  synthetic
IDTDGDT

SEQ ID NO: 79 - DNA, 42 bp, Artificial Sequence
  synthetic
gcaagatggccttggagtggtttctatggtgcttttgatatc

SEQ ID NO: 80 - protein, 14 aa, Artificial Sequence
  synthetic
ARWPWSGFYGAFDI

SEQ ID NO: 81 - DNA, 366 bp, Artificial Sequence
  synthetic
caggtgcagctgcaggagtcgggcccaggactggtgaagccttcacagaccctgtccctcacctgcactgtctctggtggctccatcagcagtggtaattactactggaactggatccgccaacagccaggagagggcctggagtggattgcttacatctatcacaatggggtcaccaacttcaatccgtccctcaagagtcgacttactatatcagtagacacgtctaagactcagttctccctgaagttgaggtctgtgactgccgcggacacggccgtttattactgtgcgagatcaggcagctggttcgagaactggtacttcgatctctggggccgtggcaccctggtcactgtctcctca

SEQ ID NO: 82 - protein, 122 aa, Artificial Sequence
  synthetic
QVQLQESGPGLVKPSQTLSLTCTVSGGSISSGNYYWNWIRQQPGEGLEWIAYIYHNGVTNFNPSLKSRLTISVDTSKTQFSLKLRSVTAADTAVYYCARSGSWFENWYFDLWGRGTLVTVSS

SEQ ID NO: 83 - DNA, 30 bp, Artificial Sequence
  synthetic
ggtggctccatcagcagtggtaattactac

SEQ ID NO: 84 - protein, 10 aa, Artificial Sequence
  synthetic
GGSISSGNYY

SEQ ID NO: 85 - DNA, 21 bp, Artificial Sequence
  synthetic
atctatcacaatggggtcacc

SEQ ID NO: 86 - protein, 7 aa, Artificial Sequence
  synthetic
IYHNGVT

SEQ ID NO: 87 - DNA, 42 bp, Artificial Sequence
  synthetic
gcgagatcaggcagctggttcgagaactggtacttcgatctc

SEQ ID NO: 88 - protein, 14 aa, Artificial Sequence
  synthetic
ARSGSWFENWYFDL

SEQ ID NO: 89 - DNA, 324 bp, Artificial Sequence
  synthetic
gaaattgtgttgacgcagtctccaggcaccctgtctttgtctccaggggaaagagccaccctctcctgcagggccagtcagagtgttagcagcagctacttagcctggtaccagcagaaacctggccaggctcccaggctcctcatctatggtgcatccagcagggccactggcatcccagacaggttcagtggcagtgggtctgggacagacttcactctcaccatcagcagactggagcctgaagattttgcagtgtattactgtcagcagtatggtagctcaccttggacgttcggccaagggaccaaggtggaaatcaaa

SEQ ID NO: 90 - protein, 108 aa, Artificial Sequence
  synthetic
EIVLTQSPGTLSLSPGERATLSCRASQSVSSSYLAWYQQKPGQAPRLLIYGASSRATGIPDRFSGSGSGTDFTLTISRLEPEDFAVYYCQQYGSSPWTFGQGTKVEIK

SEQ ID NO: 91 - DNA, 21 bp, Artificial Sequence
  synthetic
cagagtgttagcagcagctac

SEQ ID NO: 92 - protein, 7 aa, Artificial Sequence
  synthetic
QSVSSSY

SEQ ID NO: 93 - DNA, 9 bp, Artificial Sequence
  synthetic
ggtgcatcc

SEQ ID NO: 94 - protein, 3 aa, Artificial Sequence
  synthetic
GAS

SEQ ID NO: 95 - DNA, 27 bp, Artificial Sequence
  synthetic
cagcagtatggtagctcaccttggacg

SEQ ID NO: 96 - protein, 9 aa, Artificial Sequence
  synthetic
QQYGSSPWT

SEQ ID NO: 97 - DNA, 360 bp, Artificial Sequence
  synthetic
caggtgcagctgcaggagtcgggcccaggactggtgaagccttcggagaccctgtccctcacctgcactgtctctggtggctccatcagtaattcctactggagctggatccggcagcccccagggaagggactggagtggattggatatgtctattcccgtgggaacaccaagtacaacccctccctcacgagtcgagtcaccatgtcatttgacacgtccaagaaccagttctccctgaaactgaggtctgtgaccgccgcagacacggccgtgtattactgtgcgagaagcagcagctggtacgaggactggtacttcgatctctggggccgtggcaccctggtcactgtctcctca

SEQ ID NO: 98 - protein, 120 aa, Artificial Sequence
  synthetic
QVQLQESGPGLVKPSETLSLTCTVSGGSISNSYWSWIRQPPGKGLEWIGYVYSRGNTKYNPSLTSRVTMSFDTSKNQFSLKLRSVTAADTAVYYCARSSSWYEDWYFDLWGRGTLVTVSS

SEQ ID NO: 99 - DNA, 24 bp, Artificial Sequence
  synthetic
ggtggctccatcagtaattcctac

SEQ ID NO: 100 - protein, 8 aa, Artificial Sequence
  synthetic
GGSISNSY

SEQ ID NO: 101 - DNA, 21 bp, Artificial Sequence
  synthetic
gtctattcccgtgggaacacc

SEQ ID NO: 102 - protein, 7 aa, Artificial Sequence
  synthetic
VYSRGNT

SEQ ID NO: 103 - DNA, 42 bp, Artificial Sequence
  synthetic
gcgagaagcagcagctggtacgaggactggtacttcgatctc

SEQ ID NO: 104 - protein, 14 aa, Artificial Sequence
  synthetic
ARSSSWYEDWYFDL

SEQ ID NO: 105 - DNA, 354 bp, Artificial Sequence
  synthetic
caggtgcagctacagcagtggggcgcagggctgtttaagccttcggagaccctgtccctcacctgcgatgtctatggtgggtccttcagaggttattattggagttggatccgccagcccccagggaaggggctggagtggattggggaaatcagttatagtggtttcaccaattacaacccgtccctcaagagtcgagtcatcatatcaatagatacgtccaagaaccagttctccctgaagatgagctctgtgaccgccgcggacacggctgtttattactgtgcgagagttacctatggttatgggacctttgattattggggccagggaaccctggtcaccgtctcctca

SEQ ID NO: 106 - protein, 118 aa, Artificial Sequence
  synthetic
QVQLQQWGAGLFKPSETLSLTCDVYGGSFRGYYWSWIRQPPGKGLEWIGEISYSGFTNYNPSLKSRVIISIDTSKNQFSLKMSSVTAADTAVYYCARVTYGYGTFDYWGQGTLVTVSS

SEQ ID NO: 107 - DNA, 24 bp, Artificial Sequence
  synthetic
ggtgggtccttcagaggttattat

SEQ ID NO: 108 - protein, 8 aa, Artificial Sequence
  synthetic
GGSFRGYY

SEQ ID NO: 109 - DNA, 21 bp, Artificial Sequence
  synthetic
atcagttatagtggtttcacc

SEQ ID NO: 110 - protein, 7 aa, Artificial Sequence
  synthetic
ISYSGFT

SEQ ID NO: 111 - DNA, 36 bp, Artificial Sequence
  synthetic
gcgagagttacctatggttatgggacctttgattat

SEQ ID NO: 112 - protein, 12 aa, Artificial Sequence
  synthetic
ARVTYGYGTFDY

SEQ ID NO: 113 - protein, 1165 aa, Artificial Sequence
  hLEPR Accession No P48357
MICQKFCVVLLHWEFIYVITAFNLSYPITPWRFKLSCMPPNSTYDYFLLPAGLSKNTSNSNGHYETAVEPKFNSSGTHFSNLSKTTFHCCFRSEQDRNCSLCADNIEGKTFVSTVNSLVFQQIDANWNIQCWLKGDLKLFICYVESLFKNLFRNYNYKVHLLYVLPEVLEDSPLVPQKGSFQMVHCNCSVHECCECLVPVPTAKLNDTLLMCLKITSGGVIFQSPLMSVQPINMVKPDPPLGLHMEITDDGNLKISWSSPPLVPFPLQYQVKYSENSTTVIREADKIVSATSLLVDSILPGSSYEVQVRGKRLDGPGIWSDWSTPRVFTTQDVIYFPPKILTSVGSNVSFHCIYKKENKIVPSKEIVWWMNLAEKIPQSQYDVVSDHVSKVTFFNLNETKPRGKFTYDAVYCCNEHECHHRYAELYVIDVNINISCETDGYLTKMTCRWSTSTIQSLAESTLQLRYHRSSLYCSDIPSIHPISEPKDCYLQSDGFYECIFQPIFLLSGYTMWIRINHSLGSLDSPPTCVLPDSVVKPLPPSSVKAEITINIGLLKISWEKPVFPENNLQFQIRYGLSGKEVQWKMYEVYDAKSKSVSLPVPDLCAVYAVQVRCKRLDGLGYWSNWSNPAYTVVMDIKVPMRGPEFWRIINGDTMKKEKNVTLLWKPLMKNDSLCSVQRYVINHHTSCNGTWSEDVGNHTKFTFLWTEQAHTVTVLAINSIGASVANFNLTFSWPMSKVNIVQSLSAYPLNSSCVIVSWILSPSDYKLMYFIIEWKNLNEDGEIKWLRISSSVKKYYIHDHFIPIEKYQFSLYPIFMEGVGKPKIINSFTQDDIEKHQSDAGLYVIVPVIISSSILLLGTLLISHQRMKKLFWEDVPNPKNCSWAQGLNFQKPETFEHLFIKHTASVTCGPLLLEPETISEDISVDTSWKNKDEMMPTTVVSLLSTTDLEKGSVCISDQFNSVNFSEAEGTEVTYEDESQRQPFVKYATLISNSKPSETGEEQGLINSSVTKCFSSKNSPLKDSFSNSSWEIEAQAFFILSDQHPNIISPHLTFSEGLDELLKLEGNFPEENNDKKSIYYLGVTSIKKRESGVLLTDKSRVSCPFPAPCLFTDIRVLQDSCSHFVENNINLGTSSKKTFASYMPQFQTCSTQTHKIMENKMCDLTV

SEQ ID NO: 114 - protein, 846 aa, Artificial Sequence
  hLEPR.mmh aa 1-818: F22-D839 of P48357 aa 819-846: myc-myc-hexahistidine tag
FNLSYPITPWRFKLSCMPPNSTYDYFLLPAGLSKNTSNSNGHYETAVEPKFNSSGTHFSNLSKTTFHCCFRSEQDRNCSLCADNIEGKTFVSTVNSLVFQQIDANWNIQCWLKGDLKLFICYVESLFKNLFRNYNYKVHLLYVLPEVLEDSPLVPQKGSFQMVHCNCSVHECCECLVPVPTAKLNDTLLMCLKITSGGVIFQSPLMSVQPINMVKPDPPLGLHMEITDDGNLKISWSSPPLVPFPLQYQVKYSENSTTVIREADKIVSATSLLVDSILPGSSYEVQVRGKRLDGPGIWSDWSTPRVFTTQDVIYFPPKILTSVGSNVSFHCIYKKENKIVPSKEIVWWMNLAEKIPQSQYDVVSDHVSKVTFFNLNETKPRGKFTYDAVYCCNEHECHHRYAELYVIDVNINISCETDGYLTKMTCRWSTSTIQSLAESTLQLRYHRSSLYCSDIPSIHPISEPKDCYLQSDGFYECIFQPIFLLSGYTMWIRINHSLGSLDSPPTCVLPDSVVKPLPPSSVKAEITINIGLLKISWEKPVFPENNLQFQIRYGLSGKEVQWKMYEVYDAKSKSVSLPVPDLCAVYAVQVRCKRLDGLGYWSNWSNPAYTVVMDIKVPMRGPEFWRIINGDTMKKEKNVTLLWKPLMKNDSLCSVQRYVINHHTSCNGTWSEDVGNHTKFTFLWTEQAHTVTVLAINSIGASVANFNLTFSWPMSKVNIVQSLSAYPLNSSCVIVSWILSPSDYKLMYFIIEWKNLNEDGEIKWLRISSSVKKYYIHDHFIPIEKYQFSLYPIFMEGVGKPKIINSFTQDDIEKHQSDEQKLISEEDLGGEQKLISEEDLHHHHHH

SEQ ID NO: 115 - protein, 1051 aa, Artificial Sequence
  hLEPR.mFc aa 1-818: F22-D839 of P48357 aa 819-1051: mouse IgG2a (E98-K330 of P01863)
FNLSYPITPWRFKLSCMPPNSTYDYFLLPAGLSKNTSNSNGHYETAVEPKFNSSGTHFSNLSKTTFHCCFRSEQDRNCSLCADNIEGKTFVSTVNSLVFQQIDANWNIQCWLKGDLKLFICYVESLFKNLFRNYNYKVHLLYVLPEVLEDSPLVPQKGSFQMVHCNCSVHECCECLVPVPTAKLNDTLLMCLKITSGGVIFQSPLMSVQPINMVKPDPPLGLHMEITDDGNLKISWSSPPLVPFPLQYQVKYSENSTTVIREADKIVSATSLLVDSILPGSSYEVQVRGKRLDGPGIWSDWSTPRVFTTQDVIYFPPKILTSVGSNVSFHCIYKKENKIVPSKEIVWWMNLAEKIPQSQYDVVSDHVSKVTFFNLNETKPRGKFTYDAVYCCNEHECHHRYAELYVIDVNINISCETDGYLTKMTCRWSTSTIQSLAESTLQLRYHRSSLYCSDIPSIHPISEPKDCYLQSDGFYECIFQPIFLLSGYTMWIRINHSLGSLDSPPTCVLPDSVVKPLPPSSVKAEITINIGLLKISWEKPVFPENNLQFQIRYGLSGKEVQWKMYEVYDAKSKSVSLPVPDLCAVYAVQVRCKRLDGLGYWSNWSNPAYTVVMDIKVPMRGPEFWRIINGDTMKKEKNVTLLWKPLMKNDSLCSVQRYVINHHTSCNGTWSEDVGNHTKFTFLWTEQAHTVTVLAINSIGASVANFNLTFSWPMSKVNIVQSLSAYPLNSSCVIVSWILSPSDYKLMYFIIEWKNLNEDGEIKWLRISSSVKKYYIHDHFIPIEKYQFSLYPIFMEGVGKPKIINSFTQDDIEKHQSDEPRGPTIKPCPPCKCPAPNLLGGPSVFIFPPKIKDVLMISLSPIVTCVVVDVSEDDPDVQISWFVNNVEVHTAQTQTHREDYNSTLRVVSALPIQHQDWMSGKEFKCKVNNKDLPAPIERTISKPKGSVRAPQVYVLPPPEEEMTKKQVTLTCMVTDFMPEDIYVEWTNNGKTELNYKNTEPVLDSDGSYFMYSKLRVEKKNWVERNSYSCSVVHEGLHNHHTTKSFSRTPGK

SEQ ID NO: 116 - protein, 1045 aa, Artificial Sequence
  hLEPR.hFc aa 1-818: F22-D839 of P48357 aa 819-1045: human IgG1 tag (D104-K330 of P01857)
FNLSYPITPWRFKLSCMPPNSTYDYFLLPAGLSKNTSNSNGHYETAVEPKFNSSGTHFSNLSKTTFHCCFRSEQDRNCSLCADNIEGKTFVSTVNSLVFQQIDANWNIQCWLKGDLKLFICYVESLFKNLFRNYNYKVHLLYVLPEVLEDSPLVPQKGSFQMVHCNCSVHECCECLVPVPTAKLNDTLLMCLKITSGGVIFQSPLMSVQPINMVKPDPPLGLHMEITDDGNLKISWSSPPLVPFPLQYQVKYSENSTTVIREADKIVSATSLLVDSILPGSSYEVQVRGKRLDGPGIWSDWSTPRVFTTQDVIYFPPKILTSVGSNVSFHCIYKKENKIVPSKEIVWWMNLAEKIPQSQYDVVSDHVSKVTFFNLNETKPRGKFTYDAVYCCNEHECHHRYAELYVIDVNINISCETDGYLTKMTCRWSTSTIQSLAESTLQLRYHRSSLYCSDIPSIHPISEPKDCYLQSDGFYECIFQPIFLLSGYTMWIRINHSLGSLDSPPTCVLPDSVVKPLPPSSVKAEITINIGLLKISWEKPVFPENNLQFQIRYGLSGKEVQWKMYEVYDAKSKSVSLPVPDLCAVYAVQVRCKRLDGLGYWSNWSNPAYTVVMDIKVPMRGPEFWRIINGDTMKKEKNVTLLWKPLMKNDSLCSVQRYVINHHTSCNGTWSEDVGNHTKFTFLWTEQAHTVTVLAINSIGASVANFNLTFSWPMSKVNIVQSLSAYPLNSSCVIVSWILSPSDYKLMYFIIEWKNLNEDGEIKWLRISSSVKKYYIHDHFIPIEKYQFSLYPIFMEGVGKPKIINSFTQDDIEKHQSDDKTHTCPPCPAPELLGGPSVFLFPPKPKDTLMISRTPEVTCVVVDVSHEDPEVKFNWYVDGVEVHNAKTKPREEQYNSTYRVVSVLTVLHQDWLNGKEYKCKVSNKALPAPIEKTISKAKGQPREPQVYTLPPSRDELTKNQVSLTCLVKGFYPSDIAVEWESNGQPENNYKTTPPVLDSDGSFFLYSKLTVDKSRWQQGNVFSCSVMHEALHNHYTQKSLSLSPGK

SEQ ID NO: 117 - protein, 844 aa, Artificial Sequence
  MfLEPR.mmh aa 1-816: Macaca fascicularis F22-D837 with a T827A substitution from XP_005543194.1 aa 817-844: myc-myc-hexahistidine tag
FNLSYPITPWRFKLSCMPPNSTYDYFLLPAGLSKNTSNLNGHYETAVEFNSSDTHFSNLSKTTFHCCFRSEQDRNCSLCADNIEGKTFVSTVNSSVFQQMGANWNIQCWLKGDLKLFICYVESLFKNPFKNYKHKVHLLYVLPEVLEDSPLVPQKGSFQMVHCNCSVHERCECLVPVPTAKLNDTLLMCLKITSGGVIFQSPLMSVQPINMVKPDPPLGLRMEITDDGNLKISWSSPPLVPFPLQYEVKYSENSTTVIREADKIVSATSLLVDGILPGSSYEVQVRGKRLDGPGIWSDWSTPHVFTTQDVIYFPPKILTSVGSNVSFHCIYKNENKIVSSKKIVWWMNLAEKIPQSQYDVVSDHVSKVTFFNLNETKPRGKFTYDAVYCCNEHECHHRYAELYVIDVNINISCETDGHLTKMTCRWSTNTIQSLAGSTLQLRYRRSSLYCFDIPSIHPISKPKDCYLQSDGFYECVFQPIFLLSGYTMWIRINHPLGSLDSPPTCVLPDSVVKPLPPSSVKAEIIKNIGLLKISWEKPVFPENNLQFQIRYGLSGKEIQWKMYDVYDAKSKSVSLPVPDFCAVYAVQVRCKRSDGLGLWSNWSNPAYTVVMDIKVPMRGPEFWRIINGDTMKKEKNVTLLWKPLMKNDSLCSVQRYVINHHTSCNGTWSEDVGNHTKFTFLWTEQAHTVTVLAINSIGASVANFNLTFSWPMSKVNIVQSLSAYPLNSSCVILSWILSPSDYKLMYFIIEWKNLNEDGEIKWLRISSSVKKYYIHDHFIPIEKYQFSLYPIFMEGVGKPKIINSFAQDNTEKHQNDEQKLISEEDLGGEQKLISEEDLHHHHHH

SEQ ID NO: 118 - protein, 846 aa, Artificial Sequence
  mLEPR.mmh aa 1-818: Mouse LEPR (L22-G839 of NP_666258.2) aa 817-846: myc-myc-hexahistidine tag
LNLAYPISPWKFKLFCGPPNTTDDSFLSPAGAPNNASALKGASEAIVEAKFNSSGIYVPELSKTVFHCCFGNEQGQNCSALTDNTEGKTLASVVKASVFRQLGVNWDIECWMKGDLTLFICHMEPLPKNPFKNYDSKVHLLYDLPEVIDDSPLPPLKDSFQTVQCNCSLRGCECHVPVPRAKLNYALLMYLEITSAGVSFQSPLMSLQPMLVVKPDPPLGLHMEVTDDGNLKISWDSQTMAPFPLQYQVKYLENSTIVREAAEIVSATSLLVDSVLPGSSYEVQVRSKRLDGSGVWSDWSSPQVFTTQDVVYFPPKILTSVGSNASFHCIYKNENQIISSKQIVWWRNLAEKIPEIQYSIVSDRVSKVTFSNLKATRPRGKFTYDAVYCCNEQACHHRYAELYVIDVNINISCETDGYLTKMTCRWSPSTIQSLVGSTVQLRYHRRSLYCPDSPSIHPTSEPKNCVLQRDGFYECVFQPIFLLSGYTMWIRINHSLGSLDSPPTCVLPDSVVKPLPPSNVKAEITVNTGLLKVSWEKPVFPENNLQFQIRYGLSGKEIQWKTHEVFDAKSKSASLLVSDLCAVYVVQVRCRRLDGLGYWSNWSSPAYTLVMDVKVPMRGPEFWRKMDGDVTKKERNVTLLWKPLTKNDSLCSVRRYVVKHRTAHNGTWSEDVGNRTNLTFLWTEPAHTVTVLAVNSLGASLVNFNLTFSWPMSKVSAVESLSAYPLSSSCVILSWTLSPDDYSLLYLVIEWKILNEDDGMKWLRIPSNVKKFYIHDNFIPIEKYQFSLYPVFMEGVGKPKIINGFTKDAIDKQQNDAGEQKLISEEDLGGEQKLISEEDLHHHHHH

SEQ ID NO: 119 - protein, 846 aa, Artificial Sequence
  rLEPR.mmh aa 1-818: Rat LEPR (L22-G839 of NP_036728.1) aa 819-846: myc-myc-hexahistidine tag
LNLAYPTSPWRFKLFCAPPSTTDDSFLSPAGVPNNTSSLKGASEALVEAKFNSTGIYVSELSKTIFHCCFGNEQGQNCSALTGNTEGKTLASVVKPLVFRQLGVNWDIECWMKGDLTLFICHMEPLLKNPFKNYDSKVHLLYDLPEVIDDLPLPPLKDSFQTVQCNCSVRECECHVPVPRAKVNYALLMYLEITSAGVSFQSPLMSLQPMLVVKPDPPLGLRMEVTDDGNLKISWDSQTKAPFPLQYQVKYLENSTIVREAAEIVSDTSLLVDSVLPGSSYEVQVRSKRLDGSGVWSDWSLPQLFTTQDVMYFPPKILTSVGSNASFCCIYKNENQTISSKQIVWWMNLAEKIPETQYNTVSDHISKVTFSNLKATRPRGKFTYDAVYCCNEQACHHRYAELYVIDVNINISCETDGYLTKMTCRWSPSTIQSLVGSTVQLRYHRRSLYCPDNPSIRPTSELKNCVLQTDGFYECVFQPIFLLSGYTMWIRINHSLGSLDSPPTCVLPDSVVKPLPPSNVKAEITINTGLLKVSWEKPVFPENNLQFQIRYGLNGKEIQWKTHEVFDAKSKSASLPVSDLCAVYVVQVRCRRLDGLGYWSNWSSPAYTLVMDVKVPMRGPEFWRIMDGDITKKERNVTLLWKPLMKNDSLCSVRRYVVKHRTAHNGTWSQDVGNQTNLTFLWAESAHTVTVLAINSIGASLVNFNLTFSWPMSKVNAVQSLSAYPLSSSCVILSWTLSPNDYSLLYLVIEWKNLNDDDGMKWLRIPSNVNKYYIHDNFIPIEKYQFSLYPVFMEGVGKPKIINGFTKDDIAKQQNDAGEQKLISEEDLGGEQKLISEEDLHHHHHH

SEQ ID NO: 120 - protein, 1045 aa, Artificial Sequence
  mLEPR.hFc aa 1-818: Mouse LEPR (L22-G839 of NP_666258.2) aa 819-1045: human IgG1 tag (D104-K330 of P01857)
LNLAYPISPWKFKLFCGPPNTTDDSFLSPAGAPNNASALKGASEAIVEAKFNSSGIYVPELSKTVFHCCFGNEQGQNCSALTDNTEGKTLASVVKASVFRQLGVNWDIECWMKGDLTLFICHMEPLPKNPFKNYDSKVHLLYDLPEVIDDSPLPPLKDSFQTVQCNCSLRGCECHVPVPRAKLNYALLMYLEITSAGVSFQSPLMSLQPMLVVKPDPPLGLHMEVTDDGNLKISWDSQTMAPFPLQYQVKYLENSTIVREAAEIVSATSLLVDSVLPGSSYEVQVRSKRLDGSGVWSDWSSPQVFTTQDVVYFPPKILTSVGSNASFHCIYKNENQIISSKQIVWWRNLAEKIPEIQYSIVSDRVSKVTFSNLKATRPRGKFTYDAVYCCNEQACHHRYAELYVIDVNINISCETDGYLTKMTCRWSPSTIQSLVGSTVQLRYHRRSLYCPDSPSIHPTSEPKNCVLQRDGFYECVFQPIFLLSGYTMWIRINHSLGSLDSPPTCVLPDSVVKPLPPSNVKAEITVNTGLLKVSWEKPVFPENNLQFQIRYGLSGKEIQWKTHEVFDAKSKSASLLVSDLCAVYVVQVRCRRLDGLGYWSNWSSPAYTLVMDVKVPMRGPEFWRKMDGDVTKKERNVTLLWKPLTKNDSLCSVRRYVVKHRTAHNGTWSEDVGNRTNLTFLWTEPAHTVTVLAVNSLGASLVNFNLTFSWPMSKVSAVESLSAYPLSSSCVILSWTLSPDDYSLLYLVIEWKILNEDDGMKWLRIPSNVKKFYIHDNFIPIEKYQFSLYPVFMEGVGKPKIINGFTKDAIDKQQNDAGDKTHTCPPCPAPELLGGPSVFLFPPKPKDTLMISRTPEVTCVVVDVSHEDPEVKFNWYVDGVEVHNAKTKPREEQYNSTYRVVSVLTVLHQDWLNGKEYKCKVSNKALPAPIEKTISKAKGQPREPQVYTLPPSRDELTKNQVSLTCLVKGFYPSDIAVEWESNGQPENNYKTTPPVLDSDGSFFLYSKLTVDKSRWQQGNVFSCSVMHEALHNHYTQKSLSLSPGK